European Patent Application EP 4 257 681 A1, published October 11, 2023. Title: Recombinant bacterium with a high PHA yield and the construction method thereof. Applicant: 深圳蓝晶生物科技有限公司. Application CN 2022102807310, filed March 22, 2022. The sequence listing filed with the application follows.

SEQUENCE LISTING (22 sequences)

SEQ ID NO: 1 - DNA, 1770 bp, Ralstonia eutropha
  source 1..1770: mol_type = other DNA
atggcgaccggcaaaggcgcggcagcttccacgcaggaaggcaagtcccaaccattcaaggtcacgccggggccattcgatccagccacatggctggaatggtcccgccagtggcagggcactgaaggcaacggccacgcggccgcgtccggcattccgggcctggatgcgctggcaggcgtcaagatcgcgccggcgcagctgggtgatatccagcagcgctacatgaaggacttctcagcgctgtggcaggccatggccgagggcaaggccgaggccaccggtccgctgcacgaccggcgcttcgccggcgacgcatggcgcaccaacctcccatatcgcttcgctgccgcgttctacctgctcaatgcgcgcgccttgaccgagctggccgatgccgtcgaggccgatgccaagacccgccagcgcatccgcttcgcgatctcgcaatgggtcgatgcgatgtcgcccgccaacttccttgccaccaatcccgaggcgcagcgcctgctgatcgagtcgggcggcgaatcgctgcgtgccggcgtgcgcaacatgatggaagacctgacacgcggcaagatctcgcagaccgacgagagcgcgtttgaggtcggccgcaatgtcgcggtgaccgaaggcgccgtggtcttcgagaacgagtacttccagctgttgcagtacaagccgctgaccgacaaggtgcacgcgcgcccgctgctgatggtgccgccgtgcatcaacaagtactacatcctggacctgcagccggagagctcgctggtgcgccatgtggtggagcagggacatacggtgtttctggtgtcgtggcgcaatccggacgccagcatggccggcagcacctgggacgactacatcgagcacgcggccatccgcgccatcgaagtcgcgcgcgacatcagcggccaggacaagatcaacgtgctcggcttctgcgtgggcggcaccattgtctcgaccgcgctggcggtgctggccgcgcgcggcgagcacccggccgccagcgtcacgctgctgaccacgctgctggactttgccgacacgggcatcctcgacgtctttgtcgacgagggccatgtgcagttgcgcgaggccacgctgggcggcggcgccggcgcgccgtgcgcgctgctgcgcggccttgagctggccaataccttctcgttcttgcgcccgaacgacctggtgtggaactacgtggtcgacaactacctgaagggcaacacgccggtgccgttcgacctgctgttctggaacggcgacgccaccaacctgccggggccgtggtactgctggtacctgcgccacacctacctgcagaacgagctcaaggtaccgggcaagctgaccgtgtgcggcgtgccggtggacctggccagcatcgacgtgccgacctatatctacggctcgcgcgaagaccatatcgtgccgtggaccgcggcctatgcctcgaccgcgctgctggcgaacaagctgcgcttcgtgctgggtgcgtcgggccatatcgccggtgtgatcaacccgccggccaagaacaagcgcagccactggactaacgatgcgctgccggagtcgccgcagcaatggctggccggcgccatcgagcatcacggcagctggtggccggactggaccgcatggctggccgggcaggccggcgcgaaacgcgccgcgcccgccaactatggcaatgcgcgctatcgcgcaatcgaacccgcgcctgggcgatacgtcaaagccaaggcatga

SEQ ID NO: 2 - DNA, 837 bp, Ralstonia eutropha
  source 1..837: mol_type = other DNA
atgctcgatacccttacctttggctttctcggcggcggcaacatggccaccgcactgatcggcggcctgatcgcccgcggcgtgccggccggctcgatccgcgtggtcgaccccttccccgaggcccagcaacgcctggcgcgcgacctcggcgtgcatgccgccggcgcgccggatgccgccttcggcgcctgcgacgtgctggtgctggcggtcaagccgcagcagttccgcgacgccgcggcgcagctgctgccgatcctgccggccagcggcaagggcaacctggtgatcagcgtggccgccggcatccggctgcaggacatggagcgctggctggacgggcgcgcccggctggtgcgggcgatgccgaacacgccggcgctggccggcatgggcatgaccgggctggccgcgccggccgggctgtcggccgaagaccgcgcgatcgccagcgcggtggccgaggccgtcggcaagtgcgtatgggtggatggggatgaccagatcgatgcggtcaccgccatttccggcagtgggccggcctatgtcttctactttatcgaagcgatggaacgcgccgccaccgagctgggcctgacggcggagcaaggccgcgaactggcggtagaaaccttccgtggcgctgctaccctggccgggcagtcttccgagccggtgtcgacgctgcgtgagcgcgtgacgtccaagggcggcacgacgtatgcggcgctgacggcgatggaggcttcgggcattggtgatgccttcgtgcgcgcgatgcatgctgccgcggcgcggggcaaggagatgggggcggagttcgggaaggattga

SEQ ID NO: 3 - DNA, 146 bp, Ralstonia eutropha
  source 1..146: mol_type = other DNA
atgcctccacaccgctcgtcacatcctgttgcgttcactggaatcccacgatagagtttgacctgcgagcaagctgtcaccggatgtgctttccggtctgatgagtccgtgaggacgaaacagcctctacaaataattttgtttaa

SEQ ID NO: 4 - DNA, 2025 bp, Ralstonia eutropha
  source 1..2025: mol_type = other DNA
ggtctcacaaggtggacatccttgtgcgtcatcgaggcgatgttgatccggcgcatgtcgccgtggatccgcaccatcggcggcatgtccgcggagagatgaagatcagacgccttgttcttgacagcgaaagccaatagctgcgcgatgtccatctataatgaccccaccctagttatcagtactttgcgtactttcttttgtatgttcgccggattatgtctgtaattgccgccaacttgcaagccgttcaccagcgcatcgcggcggccgcacaacaagccggcagacagcccgcggacatcgccctgctggcggtttccaagaccgttccccccgaccgcataagggccgcatacgccgccggacaggtcgctttcggcgaaaactacgtccaggaaggcgtcgacaagatcgccgcgctggccgacctgcgccaccgcctgcaatggcatttcatcggcccgctgcagagcaacaagacccgcctggtggcggagcatttcgactgggtgcacgccgtcgaccggctcaggatcgccgagcggctgtcggcccagcgcccggccggcatggccgcgctgcaggtctgcatccaggtcaatatcagcggcgaagccagcaagagcggcgtcgccccggcagaggtgcccggcctggcacatgccgtcgccgcgctgccaggcctgcgcctgcgcgggctgatggccatccccgagcccgagcacgaccccgccgcgcagcgccgcccgttcgcggccatgcgcgccatgctgcaggcgctgcgcaccgacggcctggacctcgacacgctgtcgatgggcatgtcgggcgacatggaagccgccatcgccgagggcgccacgctggtgcggatcggcaccgccattttcggagcgcgccaatacccgtagtccggcgcgcccagtccattcccttcaagccccccaacggatctccatgctcgatacccttacctttggctttctcggcggcggcaacatggccaccgcactgatcggcggcctgatcgcccgcggcgtgccggccggctcgatccgcgtggtcgaccccttccccgaggcccagcaacgcctggcgcgcgacctcggcgtgcatgccgccggcgcgccggatgccgccttcggcgcctgcgacgtgctggtgctggcggtcaagccgcagcagttccgcgacgccgcggcgcagctgctgccgatcctgccggccagcggcaagggcaacctggtgatcagcgtggccgccggcatccggctgcaggacatggagcgctggctggacgggcgcgcccggctggtgcgggcgatgccgaacacgccggcgctggccggcatgggcatgaccgggctggccgcgccggccgggctgtcggccgaagaccgcgcgatcgccagcgcggtggccgaggccgtcggcaagtgcgtatgggtggatggggatgaccagatcgatgcggtcaccgccatttccggcagtgggccggcctatgtcttctactttatcgaagcgatggaacgcgccgccaccgagctgggcctgacggcggagcaaggccgcgaactggcggtagaaaccttccgtggcgctgctaccctggccgggcagtcttccgagccggtgtcgacgctgcgtgagcgcgtgacgtccaagggcggcacgacgtatgcggcgctgacggcgatggaggcttcgggcattggtgatgccttcgtgcgcgcgatgcatgctgccgcggcgcggggcaaggagatgggggcggagttcgggaaggattgaggcgcggccaaaccgcgggcgctctgacctggccgccgccccatgtgaacgctcccctctcccgcaagcgggagaggggagaaaaccagcgggatctaatcagcgaattgcataagccaccgccgtccccgcaaacacacaggcccccagccagttgttatgccggaacgccgcgaaacaccgcatccggtcgcggtcacgaatcagcgtgtaatgatacctgagacc

SEQ ID NO: 5 - DNA, 2256 bp, synthetic construct
  source 1..2256: mol_type = other DNA
ggtctcatacccaaaaattcatccttctcgcctatgctctggggcctcggcagatgcgagcgctgcataccgtccggtaggtcgggaagcgtgcagtgccgaggcggattcccgcattgacagcgcgtgcgttgcaaggcaacaatggactcaaatgtctcggaatcgctgacgattcccaggtttctccggcaagcatagcgcatggcgtctccatgcgagaatgtcgcgcttgccggataaaaggggagccgctatcggaatggacgcaagccacggccgcagcaggtgcggtcgagggcttccagccagttccagggcagatgtgccggcagaccctcccgctttgggggaggcgcaagccgggtccattcggatagcatctccccatgcaaagtgccggccagggcaatgcccggagccggttcgaatagtgacggcagagagagacaatcaaatcatgagccaaccatcttatggcccgctgttcgaggccctggcccactacaatgacaagctgctggccatggccaaggcccagacagagcgcaccgcccaggcgctgctgcagaccaatctggacgatctgggccaggtgctggagcagggcagccagcaaccctggcagctgatccaggcccagatgaactggtggcaggatcagctcaagctgatgcagcacaccctgctcaaaagcgcaggccagccgagcgagccggtgatcaccccggagcgcagcgatcgccgcttcaaggccgaggcctggagcgaacaacccatctatgactacctcaagcagtcctacctgctcaccgccaggcacctgctggcctcggtggatgccctggagggcgtcccccagaagagccgggagcggctgcgtttcttcacccgccagtacgtctctgccatggcccccagcaacttcctggccaccaaccccgagctgctcaagctgaccctggagtccggcggccagaacctggtgcgcggactggccctcttggccgaggatctggagcgcagcgccgatcagctcaacatccgcctgaccgacgaatccgccttcgagctcgggcgggatctggccctgaccccgggccgggtggtgcagcgcaccgagctctatgagctcattcagtacagcccgactaccgagacggtgggcaagacacctgtgctgatagtgccgcccttcatcaacaagtactacatcatggacatgcggccccagaactccctggtcgcctggctggtcgcccagggccagacggtattcatgatctcctggcgcaacccgggcgtggcccaggcccaaatcgatctcgacgactacgtggtggatggcgtcatcgccgccctggacggcgtggaggcggccaccggcgagcgggaggtgcacggcatcggctactgcatcggcggcaccgccctgtcgctcgccatgggctggctggcggcgcggcgccagaagcagcgggtgcgcaccgccaccctgttcactaccctgctggacttctcccagcccggggagcttggcatcttcatccacgagcccatcatagcggcgctcgaggcgcaaaatgaggccaagggcatcatggacgggcgccagctggcggtcagcttcagcctgctgcgggagaacagcctctactggaactactacatcgacagctacctcaagggtcagagcccggtggccttcgatctgctgcactggaacagcgacagcaccaatgtggcgggcaagacccacaacagcctgctgcgccgtctctacctggagaaccagctggtgaagggggagctcaagatccgcaacacccgcatcgatctcggcaaggtgaagacccctgtgctgctggtgtcggcggtggacgatcacatcgccctctggcagggcacctggcagggcatgaagctgtttggcggggagcagcgcttcctcctggcggagtccggccacatcgccggcatcatcaacccgccggccgccaacaagtacggcttctggcacaacggggccgaggccgagagcccggagagctggctggcaggggcgacgcaccagggcggctcctggtggcccgagatgatgggctttatccagaaccgtgacgaagggtcagagcccgtccccgcgcgggtcccggaggaagggctggcccccgcccccggccactatgtcaaggtgcggctcaaccccgtgtttgcctgcccaacagaggaggacgccgcatgaccgctgagacc

SEQ ID NO: 6 - DNA, 6752 bp, synthetic construct
  source 1..6752: mol_type = other DNA
cgtctcattttcgccagatatcggtagcggagtgtatactggcttactatgttggcactgatgagggtgtcagtgaagtgcttcatgtggcaggagaaaaaaggctgcaccggtgcgtcagcagaatatgtgatacaggatatattccgcttcctcgctcactgactcgctacgctcggtcgttcgactgcggcgagcggaaatggcttacgaacggggcggagatttcctggaagatgccaggaagatacttaacagggaagtgagagggccgcggcaaagccgtttttccataggctccgcccccctgacaagcatcacgaaatctgacgctcaaatcagtggtggcgaaacccgacaggactataaagataccaggcgtttcccctggcggctccctcgtgcgctctcctgttcctgcctttcggtttaccggtgtcattccgctgttatggccgcgtttgtctcattccacgcctgacactcagttccgggtaggcagttcgctccaagctggactgtatgcacgaaccccccgttcagtccgaccgctgcgccttatccggtaactatcgtcttgagtccaacccggaaagacatgcaaaagcaccactggcagcagccactggtaattgatttagaggagttagtcttgaagtcatgcgccggttaaggctaaactgaaaggacaagttttggtgactgcgctcctccaagccagttacctcggttcaaagagttggtagctcagagaaccttcgaaaaaccgccctgcaaggcggttttttcgttttcagagcaagagattacgcgcagaccaaaacgatctcaagaagatcatcttattaaagggtccccaataattacgatttaaattggatgaatgtcagctactgggctatctggacaagggaaaacgcaagcgcaaagagaaagcaggtagcttgcagtgggcttacatggcgatagctagactgggcggttttatggacagcaagcgaaccggaattgccagctggggcgccctctggtaaggttgggaagccctgcaaagtaaactggatggctttcttgccgccaaggatctgatggcgcaggggatcaagatctgatcaagagacaggatgaggatcgtttcgcatgattgaacaagatggattgcacgcaggttctccggccgcttgggtggagaggctattcggctatgactgggcacaacagacaatcggctgctctgatgccgccgtgttccggctgtcagcgcaggggcgcccggttctttttgtcaagaccgacctgtccggtgccctgaatgaactgcaggacgaggcagcgcggctatcgtggctggccacgacgggcgttccttgcgcagctgtgctcgacgttgtcactgaagcgggaagggactggctgctattgggcgaagtgccggggcaggatctcctgtcatctcaccttgctcctgccgagaaagtatccatcatggctgatgcaatgcggcggctgcatacgcttgatccggctacctgcccattcgaccaccaagcgaaacatcgcatcgagcgagcacgtactcggatggaagccggtcttgtcgatcaggatgatctggacgaagagcatcaggggctcgcgccagccgaactgttcgccaggctcaaggcgcgcatgcccgacggcgaggatctcgtcgtgacccatggcgatgcctgcttgccgaatatcatggtggaaaatggccgcttttctggattcatcgactgtggccggctgggtgtggcggaccgctatcaggacatagcgttggctacccgtgatattgctgaagagcttggcggcgaatgggctgaccgcttcctcgtgctttacggtatcgccgctcccgattcgcagcgcatcgccttctatcgccttcttgacgagttcttctgatcaatttccgagaatgacagttctcagaaattgatttgacttttgtccttttccgctgcataaccctgcttcggggtcattatagcgattttttcggtatatccatcctttttcgcacgatatacaggattttgccaaagggttcgtgtagactttccttggtgtatccaacggcgtcagccgggcaggataggtgaagtaggcccacccgcgagcgggtgttccttcttcactgtcccttattcgcacctggcggtgctcaacgggaatcctgctctgcgaggctggccgtaggccggccgcgatgcaggtggctgctgaacccccagccggaactgaccccacaaggccctgtacacgcctcaaaaggacgggagtgggacagcgtagccatagtccgagccgaagagacaatcgttcccgacagcgaaagcccagaaagcgaagaaaggcgcctcttctacgtcgccgtcacgcgcgccagggattgcctgtttatctcaacggcgaagaagaacccgacctcgcgcttcgtccttgaggctggcctaagccttacttcctgaggcgcgcattctttgtgcgttatatggcactttcgtagaattcctcgccttttactttaacaacgacccgtaagtaccgggggaacagctcgatctctcgggtacaacaggcacaaagttaacttgcgtatacgtctaagggccgctaaccttcacggcaacgcaaccgcggacgtcatttttgccgaaaacggttgcacgatccaccggcggttccggtgaacagcttaaaggtttttgaaccgaatggatatcaagctagcccaccccagcaagacgacgcctgaggatttgaagcagttggcaaatctctccgcggtgatgctgcagaaaattcgggatgagatgctggagccatttcctcggaaggaagccccgctgatcccgtctggccgcctacaagaattgtgtggcatcgacaaaacgcggatgaaccggtccctcaaaaagggggatctccctcagggccagcaatcgcgacccggtgcagtgcgctatttcagcctcagcgaggcaatgcaatggatccgagcggaacttaagcctgtcccgcgaaggggaccaggtaaagtcattgcagttgcgaacttcaagggcggtgtcacgaagaccactatgtccaccctcctctgccagggcttgagtctgcggcgaggtcggaaggtgtgccacgttgatctggatccgcagggaagcgcaaccacgctgtatggcatcaatccacatgccgaggtgtcgtccgaaaacaccattatgccgctcatcgaggcgtatttggcgggcgagtccttcgatatgcgagggcttcctcaggagacttactggcctaacctggatttgattccttcgtctactgagcttttcaacgcggagtttatgcttccggctcgggcgacggcagaggaaggccatattccgttcgagcgcgtgttaagtaacggcctcgattcgttgaaagacgaatatgactacatcatcctcgacacggctcctaccctcagctacctgaccatcaacgcgattttcgctgccgatggcgtcatcgtaccggtggtcccggacaccttggctttcgcgtctatggtccagttctggcaactcttctcggacctagtaacaggcatggaagagcagagcgagggatctaaaaaggagttcgactttctcgatgttctcatgacacgcatggagaaaaagaacgctcctcgcctggtggcagactggattcgcggcgtctatgggtcgcgcgtgctgccgattgagatccctgagacggacctcgcccgtaacagcagcattcaatttcgcacggtctatgacctctcctctagcgaggcgaacaccgagacgatgcgacgcattcgccaaccctgcgatgagtttgtcgactatgtggacgacaaggtcagcgcgctttggcaaggaattgaagaatgagtttgagagaaaagcttgccgcaaaggctgggaacatcaaggtcacggcggaagacttggagaaagccgctgcgcgcggtccgcaagcgccgcgaactgcgcccggtcagttaatgcatatgcaagggaaggttgagcgacaggctaacgagatcgcgcaactaagagcagaacttgagtcggcccgcgtcagcggcggcgcagtggatgtgcctatcgaccaactgcatgaggtcccaggccgcagacgcttcatgcctcccgagaagtatgtcgaattgagggaaaacctcaggcacaacaagctcgttcatcctgtgattgtatgccctcggcctgcgggaggcttcgagattgtctccgggcatcaccggacagacgcgtaccgcgagcttgggcgcgatcacatacgctgcgtgctcggcgaacttagttcagacgaggctgacacgggcgcgttctacgcgaaccttatgcagtcagatttaacggatttcgagaagtttcggaagttcgacgaactgctgcttcgcagcccagacaagactcaagccgcaatagctgaacaggctggtgtacctgtctcgactctctcagagattttgtcgttccggaacttgcctcccgaggtcctaagccttctcgatagccgcccagacctgctcgggtcgaatgctggcgccgagttggcaagggcgaccaaagacggtcgcggggatcgggtcgtcgaagcggttaagttgttggccgagaagaagatcgatcaacagcaggccgtacggatgactaaggccgagcaggttaagaccaggcctgccgcatctaccggcttcaaaatcaaggcgggaaaggcgacttggtgcgatgttcgtatcgcaaagaaagtcatgcgcattgagttccgcagcgaggaagaagcggaagcggcccaatcggccattcgcgaacatctggaagggttagctaaagctgcgtcggaagacgcaaaaagctaagtgcttgttttttaaggacttcgtactacgaatcgaggttttaagccatgtctagactgtaatcctacaaaaacaaaagcccacggcggcaaccgtgggcttttgagaacttcaagctgaccagtttcccggccgctacacaccgaagccactcgacatggattcgttagtcggagtgtagcggaacgcgaacctgagtcaagcgacttcaaccattttttacgaatgggaaggtcatatgactttcgcgcaacgctccgttgctggcgaggatgttgctcgcccacaaaaacaccttaaccagacagacgctctgattgctccggcgcccaagcgcctcaaacgcaagactatcgaagcagtcgagcgcgcaactcgaatcgtcgggatcgggcgtagcgcccgatcagctcttgccgccctcgcccgcacggcgaataacgatgaccccaccggtaagatctttaagcaccgggaaacgctttgtgccgaaaccggaatgtcgccggctacttggtaccgtgctcaacgagaactgctcgacttgggcctaattaccgtcgacgttcaagttcggaagcgatttggccgattcgcaggagcctacatttacctgacggaaaaagcgacggagatgctcggcttaagctcgcgaaaagaagaagaaaccacgggtacgggcgaggacgacacagcgcagctcggcgagccggccgttccaccaccctcttctatggcgcaaccgtctctcaaaacgagagtcctgtttacagaagatcgtgtcccatactcctttcaaaaaagacagcaggatcggctcccccaggacctgacacgtctgcgcggcctgggtcttgatgtaaatttaattttttggttgatgcgaaaggctaaagagcaaggccactttctctcagatgtcgtaagcgcgacatgggagagtcttgcgaaagcacgcgtgccaaaagcgtatctgcttgccctactcaccgcccgcaccgatttcagtgctgtctgcaaagcaaaggcactcaaagaagacaaagcccgaatccaagtgcaggaccgcgatttcgtgcgttcgatactcgcaggggcagcgcggcagtgtttcgtggacgaaaaaggcaaccatttcgaagtcgaaagcgacggaagctcagtgcttgtcaccgaggtccaaagtgcggtcacttcccgcttggtaggaacttccctcgccgaatttgcaaggcgactacacgctggtgcgtaccagaaagctgaggtctacgctgctccccagagagcaagcggccggctcgagaaacggggaaaggaggcggcttcgacgttatcggcgttgcgagcgatgctgcgcgaccgcaggtcagccaacgcggcaaacacgacgaacaatgctcatgccatggcctagggtgtgttttgcgctgaaagtctagggcggcggatttgtcctactcaggagagcgttcaccgacaaacaacagataaaacgaaaggcccagtctttcgactgagcctttcgttttatttgatgcctttaattaaagcggataacaatttcacacaggagagtgaagagcttttgctcttcatccaagcgagaccaaaaggtctcgccgcgacccattaccgcctttgagtgagcgtcgtgactgggaaaaccctggcgactagtcttggactcctgttgatagatccagtaatgacctcagaactccatctggatttgttcagaacgctcggttgccgccgggcgttttttattggtgagaatccagtcaatttccgagaatgacagttctcagaaattgaa

SEQ ID NO: 7 - DNA, 1825 bp, synthetic construct
  source 1..1825: mol_type = other DNA
ggcagagagacaatcaaatcatgagccaaccatcttatggcccgctgttcgaggccctggcccactacaatgacaagctgctggccatggccaaggcccagacagagcgcaccgcccaggcgctgctgcagaccaatctggacgatctgggccaggtgctggagcagggcagccagcaaccctggcagctgatccaggcccagatgaactggtggcaggatcagctcaagctgatgcagcacaccctgctcaaaagcgcaggccagccgagcgagccggtgatcaccccggagcgcagcgatcgccgcttcaaggccgaggcctggagcgaacaacccatctatgactacctcaagcagtcctacctgctcaccgccaggcacctgctggcctcggtggatgccctggagggcgtcccccagaagagccgggagcggctgcgtttcttcacccgccagtacgtctctgccatggcccccagcaacttcctggccaccaaccccgagctgctcaagctgaccctggagtccggcggccagaacctggtgcgcggactggccctcttggccgaggatctggagcgcagcgccgatcagctcaacatccgcctgaccgacgaatccgccttcgagctcgggcgggatctggccctgaccccgggccgggtggtgcagcgcaccgagctctatgagctcattcagtacagcccgactaccgagacggtgggcaagacacctgtgctgatagtgccgcccttcatcaacaagtactacatcatggacatgcggccccagaactccctggtcgcctggctggtcgcccagggccagacggtattcatgatctcctggcgcaacccgggcgtggcccaggcccaaatcgatctcgacgactacgtggtggatggcgtcatcgccgccctggacggcgtggaggcggccaccggcgagcgggaggtgcacggcatcggctactgcatcggcggcaccgccctgtcgctcgccatgggctggctggcggcgcggcgccagaagcagcgggtgcgcaccgccaccctgttcactaccctgctggacttctcccagcccggggagcttggcatcttcatccacgagcccatcatagcggcgctcgaggcgcaaaatgaggccaagggcatcatggacgggcgccagctggcggtcagcttcagcctgctgcgggagaacagcctctactggaactactacatcgacagctacctcaagggtcagagcccggtggccttcgatctgctgcactggaacagcgacagcaccaatgtggcgggcaagacccacaacagcctgctgcgccgtctctacctggagaaccagctggtgaagggggagctcaagatccgcaacacccgcatcgatctcggcaaggtgaagacccctgtgctgctggtgtcggcggtggacgatcacatcgccctctggcagggcacctggcagggcatgaagctgtttggcggggagcagcgcttcctcctggcggagtccggccacatcgccggcatcatcaacccgccggccgccaacaagtacggcttctggcacaacggggccgaggccgagagcccggagagctggctggcaggggcgacgcaccagggcggctcctggtggcccgagatgatgggctttatccagaaccgtgacgaagggtcagagcccgtccccgcgcgggtcccggaggaagggctggcccccgcccccggccactatgtcaaggtgcggctcaaccccgtgtttgcctgcccaacagaggaggacgccgcatgacgcttgcatgagtgccggcg

SEQ ID NO: 8 - DNA, 146 bp, synthetic construct
  source 1..146: mol_type = other DNA
atgcctccacaccgctcgtcacatcctgttgcgttcactggaatcccagtatacagtttgacctgcgagcaagctgtcaccggatgtgctttccggtctgatgagtccgtgaggacgaaacagcctctacaaataattttgtttaa

SEQ ID NO: 9 - DNA, 146 bp, synthetic construct
  source 1..146: mol_type = other DNA
atgcctccacaccgctcgtcacatcctgttgcgttcactggaatcccagtatagcatttgacctgcgagcaagctgtcaccggatgtgctttccggtctgatgagtccgtgaggacgaaacagcctctacaaataattttgtttaa

SEQ ID NO: 10 - DNA, 146 bp, synthetic construct
  source 1..146: mol_type = other DNA
atgcctccacaccgctcgtcacatcctgttgcgttcactggaatcccagtataccctttgacctgcgagcaagctgtcaccggatgtgctttccggtctgatgagtccgtgaggacgaaacagcctctacaaataattttgtttaa

SEQ ID NO: 11 - DNA, 40 bp, synthetic construct
  source 1..40: mol_type = other DNA
tggtacccggccaagtctgcctacgtccaggaaggcgtcg

SEQ ID NO: 12 - DNA, 40 bp, synthetic construct
  source 1..40: mol_type = other DNA
cggtttggccgcgcctcaatatcgagcatggagatccgtt

SEQ ID NO: 13 - DNA, 38 bp, synthetic construct
  source 1..38: mol_type = other DNA
aacggatctccatgctcgatattgaggcgcggccaaac

SEQ ID NO: 14 - DNA, 38 bp, synthetic construct
  source 1..38: mol_type = other DNA
caggatgtgacgagcggtgcccgttcttcaagcgcttc

SEQ ID NO: 15 - DNA, 19 bp, synthetic construct
  source 1..19: mol_type = other DNA
ctggcggtttccaagaccg

SEQ ID NO: 16 - DNA, 19 bp, synthetic construct
  source 1..19: mol_type = other DNA
gtgttgccgctcaatgcgc

SEQ ID NO: 17 - DNA, 40 bp, synthetic construct
  source 1..40: mol_type = other DNA
gctgggccgccgaagtgagcttcgacggcgtcttcgttcc

SEQ ID NO: 18 - DNA, 38 bp, synthetic construct
  source 1..38: mol_type = other DNA
cgagcggtgtggaggcatctattcagtcagggatgcct

SEQ ID NO: 19 - DNA, 43 bp, synthetic construct
  source 1..43: mol_type = other DNA
ctacaaataattttgtttaactgactgaataggaagagcaagc

SEQ ID NO: 20 - DNA, 41 bp, synthetic construct
  source 1..41: mol_type = other DNA
ccctgatttccataaggcgccgcacgccgcgcggtgacgac

SEQ ID NO: 21 - DNA, 18 bp, synthetic construct
  source 1..18: mol_type = other DNA
ttcgtggtctcggccgat

SEQ ID NO: 22 - DNA, 19 bp, synthetic construct
  source 1..19: mol_type = other DNA
caaagtcactgggttcccg